European Patent Specification EP 3 922 649 B1, published January 17, 2024. Title: ANTI-HtrA1 ANTIBODIES AND METHODS OF USE THEREOF. Applicant: F. Hoffmann-La Roche AG. The sequence listing filed with the application follows.

SEQUENCE LISTING (160 sequences)

SEQ ID NO: 1 - protein, 5 aa, Artificial Sequence
  Synthetic Construct
  MISC_FEATURE (4)..(4): Xaa is Met or Leu
DSEXH

SEQ ID NO: 2 - protein, 17 aa, Artificial Sequence
  Synthetic Construct
  MISC_FEATURE (7)..(7): Xaa is Glu or Asp
GVDPETXGAAYNQKFKG

SEQ ID NO: 3 - protein, 10 aa, Artificial Sequence
  Synthetic Construct
GYDYDYALDY

SEQ ID NO: 4 - protein, 10 aa, Artificial Sequence
  Synthetic Construct
  MISC_FEATURE (7)..(7): Xaa is Glu or Asn
RASSSVXFIH

SEQ ID NO: 5 - protein, 7 aa, Artificial Sequence
  Synthetic Construct
  MISC_FEATURE (4)..(4): Xaa is Asn, His or Glu
ATSXLAS

SEQ ID NO: 6 - protein, 9 aa, Artificial Sequence
  Synthetic Construct
  MISC_FEATURE (4)..(4): Xaa is Ser or Tyr
  MISC_FEATURE (6)..(6): Xaa is Ala or Asn
QQWXSXPWT

SEQ ID NO: 7 - protein, 5 aa, Artificial Sequence
  Synthetic Construct
DSEMH

SEQ ID NO: 8 - protein, 17 aa, Artificial Sequence
  Synthetic Construct
GVDPETEGAAYNQKFKG

SEQ ID NO: 9 - protein, 10 aa, Artificial Sequence
  Synthetic Construct
RASSSVEFIH

SEQ ID NO: 10 - protein, 7 aa, Artificial Sequence
  Synthetic Construct
ATSNLAS

SEQ ID NO: 11 - protein, 9 aa, Artificial Sequence
  Synthetic Construct
QQWSSAPWT

SEQ ID NO: 12 - protein, 30 aa, Artificial Sequence
  Synthetic Construct
  MISC_FEATURE (28)..(28): Xaa is Lys or Thr
  MISC_FEATURE (30)..(30): Xaa is Thr, Lys, or Arg
EVQLVQSGAEVKKPGASVKVSCKASGYXFX

SEQ ID NO: 13 - protein, 14 aa, Artificial Sequence
  Synthetic Construct
WVRQAPGQGLEWIG

SEQ ID NO: 14 - protein, 32 aa, Artificial Sequence
  Synthetic Construct
RATITRDTSTSTAYLELSSLRSEDTAVYYCTR

SEQ ID NO: 15 - protein, 11 aa, Artificial Sequence
  Synthetic Construct
WGQGTLVTVSS

SEQ ID NO: 16 - protein, 30 aa, Artificial Sequence
  Synthetic Construct
EVQLVQSGAEVKKPGASVKVSCKASGYKFT

SEQ ID NO: 17 - protein, 23 aa, Artificial Sequence
  Synthetic Construct
DIQMTQSPSSLSASVGDRVTITC

SEQ ID NO: 18 - protein, 15 aa, Artificial Sequence
  Synthetic Construct
WYQQKPGKAPKPLIS

SEQ ID NO: 19 - protein, 32 aa, Artificial Sequence
  Synthetic Construct
GVPSRFSGSGSGTDFTLTISSLQPEDFATYYC

SEQ ID NO: 20 - protein, 10 aa, Artificial Sequence
  Synthetic Construct
FGQGTKVEIK

SEQ ID NO: 21 - protein, 119 aa, Artificial Sequence
  Synthetic Construct
EVQLVQSGAEVKKPGASVKVSCKASGYKFTDSEMHWVRQAPGQGLEWIGGVDPETEGAAYNQKFKGRATITRDTSTSTAYLELSSLRSEDTAVYYCTRGYDYDYALDYWGQGTLVTVSS

SEQ ID NO: 22 - protein, 106 aa, Artificial Sequence
  Synthetic Construct
DIQMTQSPSSLSASVGDRVTITCRASSSVEFIHWYQQKPGKAPKPLISATSNLASGVPSRFSGSGSGTDFTLTISSLQPEDFATYYCQQWSSAPWTFGQGTKVEIK

SEQ ID NO: 23 - protein, 119 aa, Artificial Sequence
  Synthetic Construct
QVQLQQSGAELVRPGASVTLSCKASGYTFTDSEMHWVKQTPVHGLEWIGGVDPETDGAAYNQKFKGKATLTADKSSSTAYMELRSLTSEDSAVYYCTRGYDYDYALDYWGQGTSVTVSS

SEQ ID NO: 24 - protein, 106 aa, Artificial Sequence
  Synthetic Construct
QIVLSQSPAILSASPGEKVTMTCRASSSVNFIHWYQQKPGSSPKPWISATSNLASGVPPRFSGSGSGTSYSLTISRVEAEDAATYYCQQWSSNPWTFGGGTKLEIK

SEQ ID NO: 25 - protein, 30 aa, Artificial Sequence
  Synthetic Construct
QVQLQQSGAELVRPGASVTLSCKASGYTFT

SEQ ID NO: 26 - protein, 14 aa, Artificial Sequence
  Synthetic Construct
WVKQTPVHGLEWIG

SEQ ID NO: 27 - protein, 32 aa, Artificial Sequence
  Synthetic Construct
KATLTADKSSSTAYMELRSLTSEDSAVYYCTR

SEQ ID NO: 28 - protein, 11 aa, Artificial Sequence
  Synthetic Construct
WGQGTSVTVSS

SEQ ID NO: 29 - protein, 23 aa, Artificial Sequence
  Synthetic Construct
NIVVTQSPASLAVSLGQRATISC

SEQ ID NO: 30 - protein, 15 aa, Artificial Sequence
  Synthetic Construct
WYQQKPGQPPKLLIY

SEQ ID NO: 31 - protein, 32 aa, Artificial Sequence
  Synthetic Construct
GVPARFSGSGSRTDFTLTIDPVEADDAATYYC

SEQ ID NO: 32 - protein, 10 aa, Artificial Sequence
  Synthetic Construct
FGGGTKLEIK

SEQ ID NO: 33-38 - skipped (6 entries)

SEQ ID NO: 39 - protein, 5 aa, Artificial Sequence
  Synthetic Construct
SYIMS

SEQ ID NO: 40 - protein, 17 aa, Artificial Sequence
  Synthetic Construct
YISNGGGTTYYSDTIKG

SEQ ID NO: 41 - protein, 12 aa, Artificial Sequence
  Synthetic Construct
QNFRSDGSSMDY

SEQ ID NO: 42 - protein, 15 aa, Artificial Sequence
  Synthetic Construct
RASESVDSYGKSFMH

SEQ ID NO: 43 - protein, 7 aa, Artificial Sequence
  Synthetic Construct
LASKLES

SEQ ID NO: 44 - protein, 9 aa, Artificial Sequence
  Synthetic Construct
QQNNEDPYT

SEQ ID NO: 45 - protein, 121 aa, Artificial Sequence
  Synthetic Construct
EVQLVESGGGLVQPGGSLRLSCAASGFTFSSYIMSWVRQAPGKGLEWVAYISNGGGTTYYSDTIKGRFTISRDNSKNTLYLQMNSLRAEDTAVYYCARQNFRSDGSSMDYWGQGTLVTVSS

SEQ ID NO: 46 - protein, 111 aa, Artificial Sequence
  Synthetic Construct
DIVMTQSPDSLAVSLGERATINCRASESVDSYGKSFMHWYQQKPGQPPKLLIYLASKLESGVPDRFSGSGSGTDFTLTISSLQAEDVAVYYCQQNNEDPYTFGQGTKVEIK

SEQ ID NO: 47 - protein, 30 aa, Artificial Sequence
  Synthetic Construct
EVQLVESGGGLVQPGGSLRLSCAASGFTFS

SEQ ID NO: 48 - protein, 14 aa, Artificial Sequence
  Synthetic Construct
WVRQAPGKGLEWVA

SEQ ID NO: 49 - protein, 32 aa, Artificial Sequence
  Synthetic Construct
RFTISRDNSKNTLYLQMNSLRAEDTAVYYCAR

SEQ ID NO: 50 - protein, 11 aa, Artificial Sequence
  Synthetic Construct
WGQGTLVTVSS

SEQ ID NO: 51 - protein, 23 aa, Artificial Sequence
  Synthetic Construct
DIVMTQSPDSLAVSLGERATINC

SEQ ID NO: 52 - protein, 15 aa, Artificial Sequence
  Synthetic Construct
WYQQKPGQPPKLLIY

SEQ ID NO: 53 - protein, 32 aa, Artificial Sequence
  Synthetic Construct
GVPDRFSGSGSGTDFTLTISSLQAEDVAVYYC

SEQ ID NO: 54 - protein, 10 aa, Artificial Sequence
  Synthetic Construct
FGQGTKVEIK

SEQ ID NO: 55 - protein, 121 aa, Artificial Sequence
  Synthetic Construct
EVKLVESGGGLVEPGGSLKLACVASGFTFSSYIMSWVRQTPEKRLEWVAYISNGGGTTYYSDTIKGRFTISRDNAKNTLYLQMSTLKSEDTAIYFCARQNFRSDGSSMDYWGQGTAVTVSS

SEQ ID NO: 56 - protein, 111 aa, Artificial Sequence
  Synthetic Construct
NIVVTQSPASLAVSLGQRATISCRASESVDSYGKSFMHWYQQKPGQPPKLLIYLASKLESGVPARFSGSGSRTDFTLTIDPVEADDAATYYCQQNNEDPYTFGGGTKLEIK

SEQ ID NO: 57 - protein, 30 aa, Artificial Sequence
  Synthetic Construct
EVKLVESGGGLVEPGGSLKLACVASGFTFS

SEQ ID NO: 58 - protein, 14 aa, Artificial Sequence
  Synthetic Construct
WVRQTPEKRLEWVA

SEQ ID NO: 59 - protein, 32 aa, Artificial Sequence
  Synthetic Construct
RFTISRDNAKNTLYLQMSTLKSEDTAIYFCAR

SEQ ID NO: 60 - protein, 11 aa, Artificial Sequence
  Synthetic Construct
WGQGTAVTVSS

SEQ ID NO: 61 - protein, 23 aa, Artificial Sequence
  Synthetic Construct
NIVVTQSPASLAVSLGQRATISC

SEQ ID NO: 62 - protein, 15 aa, Artificial Sequence
  Synthetic Construct
WYQQKPGQPPKLLIY

SEQ ID NO: 63 - protein, 32 aa, Artificial Sequence; identical to SEQ ID NO: 31
  Synthetic Construct

SEQ ID NO: 64 - protein, 10 aa, Artificial Sequence
  Synthetic Construct
FGGGTKLEIK

SEQ ID NO: 65 - protein, 121 aa, Artificial Sequence
  Synthetic Construct
EVKLVESGGGLVQPGGSLKLSCAASGFTFSSYIMSWVRQTPEKRLEWVAYISNGGGTTYYPDTIKGRFTISRDNAKNTLYLQMNTLKSEDTAIYFCARQNFRSDGSSMDYWGQGTSVTVSS

SEQ ID NO: 66 - protein, 111 aa, Artificial Sequence
  Synthetic Construct
NIVLTQSPASLAVSLGQRATISCRASESVDTSGRSFMHWYQQKPGQPPRLLIYLASKLESGVPARFSGSGSRTDFTLTIDPVEADDAATYYCQQNNEDPYTFGGGTNLEIK

SEQ ID NO: 67 - protein, 117 aa, Artificial Sequence
  Synthetic Construct
DVHLVESGGGLVRPGGSRKLSCEASGFTFSSFGMHWVRQAPEKGLEWVAFITSDSSTIYYADTVKGRFTISRDNPKNTLFLQMTSLRSEDTAMYYCTRSGDDYLDYWGQGTTLTVSS

SEQ ID NO: 68 - protein, 111 aa, Artificial Sequence
  Synthetic Construct
DIVLTQSPASLAVSLGQRATISCRASQSVSTSSSSYMHWYQQKPGQPPKVFIKYASNLESGVPARFSGSGSGTDFTLSIHPVEEEDTATYYCQHSWEIPFTFGGGTKLEIK

SEQ ID NO: 69 - protein, 119 aa, Artificial Sequence
  Synthetic Construct
EVMLVESGGGLVKPGGSLKLSCAASGFTFSSYVMSWVRQTPEKRLEWVAAISGGGDYTYYPDSLKGRFTISRDNARNTLYLQMSSLRSEDTAMYYCARVDYDEYSFEYWGQGTALTVSS

SEQ ID NO: 70 - protein, 111 aa, Artificial Sequence
  Synthetic Construct
DIVLTQSPASLAVSLGQRATISCRASESVDNYGISFMNWFQQKPGQPPKLLIYAASNQGSGVPARFSGSGSGTDFSLNIHPMEEDDTAMYFCQQSKEVPWTFGGGTKLEIK

SEQ ID NO: 71 - protein, 107 aa, Artificial Sequence
  Synthetic Construct
DIQMTQSPSSLSASVGDRVTITCRASQGISSYLAWYQQKPGKAPKLLIYAASSLQSGVPSRFSGSGSGTDFTLTISSLQPEDFATYYCQQYYSYPFTFGQGTKVEIK

SEQ ID NO: 72 - protein, 106 aa, Artificial Sequence
  Synthetic Construct
DIQMTQSPSSLSASVGDRVTITCRASSSVNFIHWYQQKPGKAPKPWISATSNLASGVPSRFSGSGSGTDFTLTISSLQPEDFATYYCQQWSSNPWTFGQGTKVEIK

SEQ ID NO: 73 - protein, 106 aa, Artificial Sequence
  Synthetic Construct
DIQMTQSPSSLSASVGDRVTITCRASSSVNFIHWYQQKPGKAPKPLISATSNLASGVPSRFSGSGSGTDFTLTISSLQPEDFATYYCQQWSSNPWTFGQGTKVEIK

SEQ ID NO: 74 - protein, 106 aa, Artificial Sequence
  Synthetic Construct
DIQMTQSPSSLSASVGDRVTITCRASSSVNFIHWYQQKPGKAPKPLISATSNLASGVPSRFSGSGSGTDFTLTISSLQPEDFATYYCQQWSSAPWTFGQGTKVEIK

SEQ ID NO: 75 - protein, 112 aa, Artificial Sequence
  Synthetic Construct
EVQLVQSGAEVKKPGASVKVSCKASGYTFTSYYIHWVRQAPGQGLEWIGWINPGSGNTNYAQKFQGRVTITRDTSTSTAYLELSSLRSEDTAVYYCARFDYWGQGTLVTVSS

SEQ ID NO: 76 - protein, 119 aa, Artificial Sequence
  Synthetic Construct
EVQLVQSGAEVKKPGASVKVSCKASGYTFTDSEMHWVRQAPGQGLEWIGGVDPETDGAAYNQKFKGRATLTADTSTSTAYLELSSLRSEDTAVYYCTRGYDYDYALDYWGQGTLVTVSS

SEQ ID NO: 77 - protein, 119 aa, Artificial Sequence
  Synthetic Construct
EVQLVQSGAEVKKPGASVKVSCKASGYTFTDSEMHWVRQAPGQGLEWIGGVDPETDGAAYNQKFKGRATITRDTSTSTAYLELSSLRSEDTAVYYCTRGYDYDYALDYWGQGTLVTVSS

SEQ ID NO: 78 - protein, 119 aa, Artificial Sequence
  Synthetic Construct
EVQLVQSGAEVKKPGASVKVSCKASGYTFTDSEMHWVRQAPGQGLEWIGGVDPETEGAAYNQKFKGRATITRDTSTSTAYLELSSLRSEDTAVYYCTRGYDYDYALDYWGQGTLVTVSS

SEQ ID NO: 79 - protein, 113 aa, Artificial Sequence
  Synthetic Construct
DIVMTQSPDSLAVSLGERATINCKSSQSVLYSSNNKNYLAWYQQKPGQPPKLLIYWASTRESGVPDRFSGSGSGTDFTLTISSLQAEDVAVYYCQQYYSTPFTFGQGTKVEIK

SEQ ID NO: 80 - protein, 112 aa, Artificial Sequence
  Synthetic Construct
EVQLVESGGGLVQPGGSLRLSCAASGFTFSSYAMSWVRQAPGKGLEWVGAISSSGSSTYYADSVKGRFTISRDNSKNTLYLQMNSLRAEDTAVYYCARFDYWGQGTLVTVSS

SEQ ID NO: 81 - protein, 106 aa, Artificial Sequence
  Synthetic Construct
DIQMTQSPSSLSASVGDRVTITCRASSRVNFIHWYQQKPGKAPKPLISATSNLASGVPSRFSGSGSGTDFTLTISSLQPEDFATYYCQQWSSNPWTFGQGTKVEIK

SEQ ID NO: 82 - protein, 106 aa, Artificial Sequence
  Synthetic Construct
DIQMTQSPSSLSASVGDRVTITCRASSSVHFIHWYQQKPGKAPKPLISATSNLASGVPSRFSGSGSGTDFTLTISSLQPEDFATYYCQQWSSNPWTFGQGTKVEIK

SEQ ID NO: 83 - protein, 106 aa, Artificial Sequence
  Synthetic Construct
DIQMTQSPSSLSASVGDRVTITCRASSSVEFIHWYQQKPGKAPKPLISATSNLASGVPSRFSGSGSGTDFTLTISSLQPEDFATYYCQQWSSNPWTFGQGTKVEIK

SEQ ID NO: 84 - protein, 106 aa, Artificial Sequence
  Synthetic Construct
DIQMTQSPSSLSASVGDRVTITCRASSSVNFIHWYQQKPGKAPKPLISATSHLASGVPSRFSGSGSGTDFTLTISSLQPEDFATYYCQQWSSNPWTFGQGTKVEIK

SEQ ID NO: 85 - protein, 106 aa, Artificial Sequence
  Synthetic Construct
DIQMTQSPSSLSASVGDRVTITCRASSSVNFIHWYQQKPGKAPKPLISATSELASGVPSRFSGSGSGTDFTLTISSLQPEDFATYYCQQWSSNPWTFGQGTKVEIK

SEQ ID NO: 86 - protein, 106 aa, Artificial Sequence
  Synthetic Construct
DIQMTQSPSSLSASVGDRVTITCRASSSVNFIHWYQQKPGKAPKPLISATSNLASGVPSRFSGSGSGTDFTLTISSLQPEDFATYYCHQWSSNPWTFGQGTKVEIK

SEQ ID NO: 87 - protein, 106 aa, Artificial Sequence
  Synthetic Construct
DIQMTQSPSSLSASVGDRVTITCRASSSVNFIHWYQQKPGKAPKPLISATSNLASGVPSRFSGSGSGTDFTLTISSLQPEDFATYYCQQWYSNPWTFGQGTKVEIK

SEQ ID NO: 88 - protein, 106 aa, Artificial Sequence
  Synthetic Construct
DIQMTQSPSSLSASVGDRVTITCRASSSVNFIHWYQQKPGKAPKPLISATSNLASGVPSRFSGSGSGTDFTLTISSLQPEDFATYYCQQWKSNPWTFGQGTKVEIK

SEQ ID NO: 89 - protein, 106 aa, Artificial Sequence
  Synthetic Construct
DIQMTQSPSSLSASVGDRVTITCRASSSVNFIHWYQQKPGKAPKPLISATSNLASGVPSRFSGSGSGTDFTLTISSLQPEDFATYYCQQWSINPWTFGQGTKVEIK

SEQ ID NO: 90 - protein, 106 aa, Artificial Sequence
  Synthetic Construct
DIQMTQSPSSLSASVGDRVTITCRASSSVNVIHWYQQKPGKAPKPLISATSNLASGVPSRFSGSGSGTDFTLTISSLQPEDFATYYCQQWKSNPWTFGQGTKVEIK

SEQ ID NO: 91 - protein, 106 aa, Artificial Sequence
  Synthetic Construct
DIQMTQSPSSLSASVGDRVTITCRASSSVEFIHWYQQKPGKAPKPLISATSNLASGVPSRFSGSGSGTDFTLTISSLQPEDFATYYCQQWYSNPWTFGQGTKVEIK

SEQ ID NO: 92 - protein, 106 aa, Artificial Sequence
  Synthetic Construct
DIQMTQSPSSLSASVGDRVTITCRASSSVEFIHWYQQKPGKAPKPLISATSHLASGVPSRFSGSGSGTDFTLTISSLQPEDFATYYCQQWYSNPWTFGQGTKVEIK

SEQ ID NO: 93 - protein, 119 aa, Artificial Sequence
  Synthetic Construct
EVQLVQSGAEVKKPGASVKVSCKASGYTFKDSEMHWVRQAPGQGLEWIGGVDPETDGAAYNQKFKGRATITRDTSTSTAYLELSSLRSEDTAVYYCTRGYDYDYALDYWGQGTLVTVSS

SEQ ID NO: 94 - protein, 119 aa, Artificial Sequence
  Synthetic Construct
EVQLVQSGAEVKKPGASVKVSCKASGYTFRDSEMHWVRQAPGQGLEWIGGVDPETDGAAYNQKFKGRATITRDTSTSTAYLELSSLRSEDTAVYYCTRGYDYDYALDYWGQGTLVTVSS

SEQ ID NO: 95 - protein, 119 aa, Artificial Sequence
  Synthetic Construct
EVQLVQSGAEVKKPGASVKVSCKASGYKFTDSEMHWVRQAPGQGLEWIGGVDPETDGAAYNQKFKGRATITRDTSTSTAYLELSSLRSEDTAVYYCTRGYDYDYALDYWGQGTLVTVSS

SEQ ID NO: 96 - protein, 119 aa, Artificial Sequence
  Synthetic Construct
EVQLVQSGAEVKKPGASVKVSCKASGYRFTDSEMHWVRQAPGQGLEWIGGVDPETDGAAYNQKFKGRATITRDTSTSTAYLELSSLRSEDTAVYYCTRGYDYDYALDYWGQGTLVTVSS

SEQ ID NO: 97 - protein, 119 aa, Artificial Sequence
  Synthetic Construct
EVQLVQSGAEVKKPGASVKVSCKASGYTFTDSELHWVRQAPGQGLEWIGGVDPETDGAAYNQKFKGRATITRDTSTSTAYLELSSLRSEDTAVYYCTRGYDYDYALDYWGQGTLVTVSS

SEQ ID NO: 98 - protein, 119 aa, Artificial Sequence
  Synthetic Construct
EVQLVQSGAEVKKPGASVKVSCKASGYTFTDSEMHWVRQAPGQGLEWIGGVDPATDGAAYNQKFKGRATITRDTSTSTAYLELSSLRSEDTAVYYCTRGYDYDYALDYWGQGTLVTVSS

SEQ ID NO: 99 - protein, 119 aa, Artificial Sequence
  Synthetic Construct
EVQLVQSGAEVKKPGASVKVSCKASGYTFTDSEMHWVRQAPGQGLEWIGGVDPETDGAFYNQKFKGRATITRDTSTSTAYLELSSLRSEDTAVYYCTRGYDYDYALDYWGQGTLVTVSS

SEQ ID NO: 100 - protein, 119 aa, Artificial Sequence
  Synthetic Construct
EVQLVQSGAEVKKPGASVKVSCKASGYTFTDSEMHWVRQAPGQGLEWIGGVDPETDGAAYNQKFKGRATITRDTSTSTAYLELSSLRSEDTAVYYCTRGYDYDIALDYWGQGTLVTVSS

SEQ ID NO: 101 - protein, 119 aa, Artificial Sequence
  Synthetic Construct
EVQLVQSGAEVKKPGASVKVSCKASGYTFTDSEMHWVRQAPGQGLEWIGGVDPETDGAAYNQKFKGRATITRDTSTSTAYLELSSLRSEDTAVYYCTRGYDYDYPLDYWGQGTLVTVSS

SEQ ID NO: 102 - protein, 119 aa, Artificial Sequence
  Synthetic Construct
EVQLVQSGAEVKKPGASVKVSCKASGYKFKDSEMHWVRQAPGQGLEWIGGVDPETDGAAYNQKFKGRATITRDTSTSTAYLELSSLRSEDTAVYYCTRGYDYDYALDYWGQGTLVTVSS

SEQ ID NO: 103 - protein, 119 aa, Artificial Sequence
  Synthetic Construct
EVQLVQSGAEVKKPGASVKVSCKASGYKFRDSEMHWVRQAPGQGLEWIGGVDPETDGAAYNQKFKGRATITRDTSTSTAYLELSSLRSEDTAVYYCTRGYDYDYALDYWGQGTLVTVSS

SEQ ID NO: 104 - protein, 119 aa, Artificial Sequence
  Synthetic Construct
EVQLVQSGAEVKKPGASVKVSCKASGYTFKDSEMHWVRQAPGQGLEWIGGVDPETEGAAYNQKFKGRATITRDTSTSTAYLELSSLRSEDTAVYYCTRGYDYDYALDYWGQGTLVTVSS

SEQ ID NO: 105 - protein, 106 aa, Artificial Sequence
  Synthetic Construct
DIQMTQSPSSLSASVGDRVTITCRASSSVEFIHWYQQKPGKAPKPLISATSNLASGVPSRFSGSGSGTDFTLTISSLQPEDFATYYCQQWYSAPWTFGQGTKVEIK

SEQ ID NO: 106 - protein, 119 aa, Artificial Sequence
  Synthetic Construct
EVQLVQSGAEVKKPGASVKVSCKASGYKFKDSEMHWVRQAPGQGLEWIGGVDPETEGAAYNQKFKGRATITRDTSTSTAYLELSSLRSEDTAVYYCTRGYDYDYALDYWGQGTLVTVSS

SEQ ID NO: 107 - protein, 119 aa, Artificial Sequence
  Synthetic Construct
EVQLVQSGAEVKKPGASVKVSCKASGYKFRDSEMHWVRQAPGQGLEWIGGVDPETEGAAYNQKFKGRATITRDTSTSTAYLELSSLRSEDTAVYYCTRGYDYDYALDYWGQGTLVTVSS

SEQ ID NO: 108 - protein, 106 aa, Artificial Sequence
  Synthetic Construct
DIQMTQSPSSLSASVGDRVTITCRASSSVEFIHWYQQKPGKAPKPLISATSHLASGVPSRFSGSGSGTDFTLTISSLQPEDFATYYCQQWYSAPWTFGQGTKVEIK

SEQ ID NO: 109 - protein, 10 aa, Artificial Sequence
  Synthetic Construct
GYTFTNYGMN

SEQ ID NO: 110 - protein, 17 aa, Artificial Sequence
  Synthetic Construct
  MISC_FEATURE (13)..(13): Xaa is Asp or Glu
WINTYTGETTYAXDFKG

SEQ ID NO: 111 - protein, 6 aa, Artificial Sequence
  Synthetic Construct
  MISC_FEATURE (5)..(5): Xaa is Asn or Ser
EGGVXN

SEQ ID NO: 112 - protein, 11 aa, Artificial Sequence
  Synthetic Construct
  MISC_FEATURE (5)..(5): Xaa is Asp or Ser
  MISC_FEATURE (7)..(7): Xaa is Asp or Glu
  MISC_FEATURE (8)..(8): Xaa is Asp or Ser
ITSTXIXXDMN

SEQ ID NO: 113 - protein, 7 aa, Artificial Sequence
  Synthetic Construct
GGNTLRP

SEQ ID NO: 114 - protein, 9 aa, Artificial Sequence
  Synthetic Construct
  MISC_FEATURE (4)..(4): Xaa is Asp or Glu
LQSXSLPYT

SEQ ID NO: 115 - protein, 17 aa, Artificial Sequence
  Synthetic Construct
WINTYTGETTYADDFKG

SEQ ID NO: 116 - protein, 6 aa, Artificial Sequence
  Synthetic Construct
EGGVNN

SEQ ID NO: 117 - protein, 11 aa, Artificial Sequence
  Synthetic Construct
ITSTDIDDDMN

SEQ ID NO: 118 - protein, 9 aa, Artificial Sequence
  Synthetic Construct
LQSDSLPYT

SEQ ID NO: 119 - protein, 115 aa, Artificial Sequence [sequence omitted]

SEQ ID NO: 120 - protein, 106 aa, Artificial Sequence
  Synthetic Construct
DIQVTQSPSSLSASVGDRVTITCITSTDIDDDMNWYQQKPGKVPKLLISGGNTLRPGVPSRFSGSGSGTDFTLTISSLQPEDVATYYCLQSDSLPYTFGQTKVEIK

SEQ ID NO: 121 - protein, 480 aa, Homo sapiens
MQIPRAALLPLLLLLLAAPASAQLSRAGRSAPLAAGCPDRCEPARCPPQPEHCEGGRARDACGCCEVCGAPEGAACGLQEGPCGEGLQCVVPFGVPASATVRRRAQAGLCVCASSEPVCGSDANTYANLCQLRAASRRSERLHRPPVIVLQRGACGQGQEDPNSLRHKYNFIADVVEKIAPAVVHIELFRKLPFSKREVPVASGSGFIVSEDGLIVTNAHVVTNKHRVKVELKNGATYEAKIKDVDEKADIALIKIDHQGKLPVLLLGRSSELRPGEFVVAIGSPFSLQNTVTTGIVSTTQRGGKELGLRNSDMDYIQTDAIINYGNSGGPLVNLDGEVIGINTLKVTAGISFAIPSDKIKKFLTESHDRQAKGKAITKKKYIGIRMMSLTSSKAKELKDRHRDFPDVISGAYIIEVIPDTPAEAGGLKENDVIISINGQSVVSANDVSDVIKRESTLNMVVRRGNEDIMITVIPEEIDP

SEQ ID NO: 122 - protein, 4 aa, Artificial Sequence
  Synthetic Construct
CPPC

SEQ ID NO: 123 - protein, 17 aa, Artificial Sequence
  Synthetic Construct
GVDPETDGAAYNQKFKG

SEQ ID NO: 124 - protein, 10 aa, Artificial Sequence
  Synthetic Construct
RASSSVNFIH

SEQ ID NO: 125 - protein, 9 aa, Artificial Sequence
  Synthetic Construct
QQWSSNPWT

SEQ ID NO: 126 - protein, 253 aa, Homo sapiens
MHSWERLAVLVLLGAAACAAPPRGRILGGREAEAHARPYMASVQLNGAHLCGGVLVAEQWVLSAAHCLEDAADGKVQVLLGAHSLSQPEPSKRLYDVLRAVPHPDSQPDTIDHDLLLLQLSEKATLGPAVRPLPWQRVDRDVAPGTLCDVAGWGIVNHAGRRPDSLQHVLLPVLDRATCNRRTHHDGAITERLMCAESNRRDSCKGDSGGPLVCGGVLEGVVTSGSRVCGNRKKPGIYTRVASYAAWIDSVLA

SEQ ID NO: 127 - protein, 115 aa, Artificial Sequence
  Synthetic Construct
QVQLQQSGAELVKPGASVKLSCKASGYTFTSYYMYWVKERPGQGLEWIGEINPTNGGTNFNEKFKSKATLTVDTSSNTAYMQLSSLTSEDSAVYYCAREGGFAYWGQGTLVTVSA

SEQ ID NO: 128 - protein, 107 aa, Artificial Sequence
  Synthetic Construct
DIVMTQSQKFMSTSVGDRVSVTCKASQNVDTDVAWFQQKPGQSPRGLIYSASSRYSGVPDRFTGSGSGTDFTLTISNVQSEDLAEYFCQQYNNYPLTFGSGTKVEIK

SEQ ID NO: 129 - protein, 464 aa, Artificial Sequence
  Synthetic Construct
MGWSCIILFLVATATGAYAQVQLQQSGAELVKPGASVKLSCKASGYTFTSYYMYWVKERPGQGLEWIGEINPTNGGTNFNEKFKSKATLTVDTSSNTAYMQLSSLTSEDSAVYYCAREGGFAYWGQGTLVTVSAASTKGPSVFPLAPSSKSTSGGTAALGCLVKDYFPEPVTVSWNSGALTSGVHTFPAVLQSSGLYSLSSVVTVPSSSLGTQTYICNVNHKPSNTKVDKKVEPKSCDKTHTCPPCPAPELLGGPSVFLFPPKPKDTLMISRTPEVTCVVVDVSHEDPEVKFNWYVDGVEVHNAKTKPREEQYNSTYRVVSVLTVLHQDWLNGKEYKCKVSNKALPAPIEKTISKAKGQPREPQVYTLPPSREEMTKNQVSLTCLVKGFYPSDIAVEWESNGQPENNYKTTPPVLDSDGSFFLYSKLTVDKSRWQQGNVFSCSVMHEALHNHYTQKSLSLSPGK

SEQ ID NO: 130 - protein, 233 aa, Artificial Sequence
  Synthetic Construct
MGWSCIILFLVATATGVHSDIVMTQSQKFMSTSVGDRVSVTCKASQNVDTDVAWFQQKPGQSPRGLIYSASSRYSGVPDRFTGSGSGTDFTLTISNVQSEDLAEYFCQQYNNYPLTFGSGTKVEIKRTVAAPSVFIFPPSDEQLKSGTASVVCLLNNFYPREAKVQWKVDNALQSGNSQESVTEQDSKDSTYSLSSTLTLSKADYEKHKVYACEVTHQGLSSPVTKSFNRGEC

SEQ ID NO: 131 - protein, 115 aa, Artificial Sequence
  Synthetic Construct
EVQLVQSGPELKKPGASVKVSCKASGYTFTNYGMNWVRQAPGQGLEWMGWINTYTGETTYAEDFKGRFVFSLDTSVSTAYLQISSLKAEDTAVYYCEREGGVNNWGQGTLVTVSS

SEQ ID NO: 132 - protein, 115 aa, Artificial Sequence
  Synthetic Construct
EVQLVQSGPELKKPGASVKVSCKASGYTFTNYGMNWVRQAPGQGLEWMGWINTYTGETTYAEDFKGRFVFSLDTSVSTAYLQISSLKAEDTAVYYCEREGGVSNWGQGTLVTVSS

SEQ ID NO: 133 - protein, 106 aa, Artificial Sequence
  Synthetic Construct
DIQVTQSPSSLSASVGDRVTITCITSTDIESDMNWYQQKPGKVPKLLISGGNTLRPGVPSRFSGSGSGTDFTLTISSLQPEDVATYYCLQSDSLPYTFGQTKVEIK

SEQ ID NO: 134 - protein, 106 aa, Artificial Sequence
  Synthetic Construct
DIQVTQSPSSLSASVGDRVTITCITSTDIESDMNWYQQKPGKVPKLLISGGNTLRPGVPSRFSGSGSGTDFTLTISSLQPEDVATYYCLQSESLPYTFGQTKVEIK

SEQ ID NO: 135 - protein, 106 aa, Artificial Sequence
  Synthetic Construct
DIQVTQSPSSLSASVGDRVTITCITSTSIESDMNWYQQKPGKVPKLLISGGNTLRPGVPSRFSGSGSGTDFTLTISSLQPEDVATYYCLQSDSLPYTFGQTKVEIK

SEQ ID NO: 136 - protein, 115 aa, Artificial Sequence
  Synthetic Construct
QIQLVQSGPELKKPGETVKISCKASGYTFTNYGMNWVKQAPGKGLKWMGWINTYTGETTYADDFKGRFVFSLETSASTAYLEINNLKNEDMATYFCEREGGVDNWGQGTTLTVSS

SEQ ID NO: 137 - protein, 107 aa, Artificial Sequence
  Synthetic Construct
ETTVTQSPASLSMAIGEKVTIRCITSTDIDDDMNWYQQKPGEPPKLLISGGNTLRPGVPSRFSSSGYGADFVFTIDNMLSEDVADYYCLQSDNLPYTFGGGTRLEIK

SEQ ID NO: 138 - skipped

SEQ ID NO: 139 - DNA, 23 bp, Artificial Sequence
  Synthetic Construct
tttyttgtccaccktggtgctgc

SEQ ID NO: 140 - DNA, 19 bp, Artificial Sequence
  Synthetic Construct
gtagaagttgttcaagaag

SEQ ID NO: 141 - DNA, 22 bp, Artificial Sequence
  Synthetic Construct
cargtcamdgtcactgrctcag

SEQ ID NO: 142 - DNA, 21 bp, Artificial Sequence
  Synthetic Construct
gaggcacctccagatgttaac

SEQ ID NO: 143 - DNA, 23 bp, Artificial Sequence
  Synthetic Construct
actgctcactggatggtgggaag

SEQ ID NO: 144 - DNA, 47 bp, Artificial Sequence
  Synthetic Construct
gcaactgcaactggagtacattcacaaattgttctctcccagtctcc

SEQ ID NO: 145 - DNA, 44 bp, Artificial Sequence
  Synthetic Construct
ggatacagttggtgcagcatcagcccgtttgatttccagcttgg

SEQ ID NO: 146 - DNA, 47 bp, Artificial Sequence
  Synthetic Construct
gcaactgcaactggagcgtacgcccaggtccagctgcagcagtctgg

SEQ ID NO: 147 - DNA, 48 bp, Artificial Sequence
  Synthetic Construct
gggcccttggtggaggctgaggagacggtgactgaggttccttgaccc

SEQ ID NO: 148 - DNA, 47 bp, Artificial Sequence
  Synthetic Construct
gcaactgcaactggagtacattcaaacattgtggtgacccaatctcc

SEQ ID NO: 149 - DNA, 44 bp, Artificial Sequence
  Synthetic Construct
ggatacagttggtgcagcatcagcccgctttatttccagcttgg

SEQ ID NO: 150 - DNA, 53 bp, Artificial Sequence
  Synthetic Construct
gcaactgcaactggagcgtacgccgaggtgaagctggtggaatctgggggagg

SEQ ID NO: 151 - DNA, 48 bp, Artificial Sequence
  Synthetic Construct
gggcccttggtggaggctgaggagacggtgactgcggttccttgaccc

SEQ ID NO: 152 - protein, 10 aa, Artificial Sequence
  Synthetic Peptide
  MISC_FEATURE: N-term Mca
  MOD_RES (9)..(9): Lys(DNP)
IRRVSYSFKK

SEQ ID NO: 153 - protein, 234 aa, Artificial Sequence
  Synthetic Construct
MKHQHQHQHQHQHQMHQSTAAAGQGQEDPNSLRHKYNFIADVVEKIAPAVVHIELYRKLPFSKREVPVASGSGFIVSEDGLIVTNAHVVTNKNRVKVELKNGATYEAKIKDVDEKADIALIKIDHQGKLPVLLLGRSSELRPGEFVVAIGSPFSLQNTVTTGIVSTTQRGGKELGLRNSDMDYIQTDAIINYGNSGGPLVNLDGEVIGINTLKVTAGISFAIPSDKIKKFLTES

SEQ ID NO: 154 - protein, 228 aa, Artificial Sequence
  Synthetic Construct
MGSSHHHHHHSSGLVPRGSHMDPNSLRHKYNFIADVVEKIAPAVVHIELFRKLPFSKREVPVASGSGFIVSEDGLIVTNAHVVTNKHRVKVELKNGATYEAKIKDVDEKADIALIKIDHQGKLPVLLLGRSSELRPGEFVVAIGSPFSLQNTVTTGIVSTTQRGGKELGLRNSDMDYIQTDAIINYGNSGGPLVNLDGEVIGINTLKVTAGISFAIPSDKIKKFLTES

SEQ ID NO: 155 - protein, 480 aa, Mus musculus
MQSLRTTLLSLLLLLLAAPSLALPSGTGRSAPAATVCPEHCDPTRCAPPPTDCEGGRVRDACGCCEVCGALEGAACGLQEGPCGEGLQCVVPFGVPASATVRRRAQAGLCVCASSEPVCGSDAKTYTNLCQLRAASRRSEKLRQPPVIVLQRGACGQGQEDPNSLRHKYNFIADVVEKIAPAVVHIELYRKLPFSKREVPVASGSGFIVSEDGLIVTNAHVVTNKNRVKVELKNGATYEAKIKDVDEKADIALIKIDHQGKLPVLLLGRSSELRPGEFVVAIGSPFSLQNTVTTGIVSTTQRGGKELGLRNSDMDYIQTDAIINYGNSGGPLVNLDGEVIGINTLKVTAGISFAIPSDKIKKFLTESHDRQAKGKAVTKKKYIGIRMMSLTSSKAKELKDRHRDFPDVLSGAYIIEVIPDTPAEAGGLKENDVIISINGQSVVTANDVSDVIKKENTLNMVVRRGNEDIVITVIPEEIDP

SEQ ID NO: 156 - protein, 104 aa, Artificial Sequence
  Synthetic Construct
ASTKGPSVFPLAPSSKSTSGGTAALGCLVKDYFPEPVTVSWNSGALTSGVHTFPAVLQSSGLYSLSSVVTVPSSSLGTQTYICNVNHKPSNTKVDKKVEPKSCD

SEQ ID NO: 157 - protein, 10 aa, Artificial Sequence
  Synthetic Construct
EPKSCDKTHT

SEQ ID NO: 158 - protein, 9 aa, Artificial Sequence
  Synthetic Construct
PAPELLGGP

SEQ ID NO: 159 - protein, 213 aa, Artificial Sequence
  Synthetic Construct
DIQMTQSPSSLSASVGDRVTITCRASSSVEFIHWYQQKPGKAPKPLISATSNLASGVPSRFSGSGSGTDFTLTISSLQPEDFATYYCQQWSSAPWTFGQGTKVEIKRTVAAPSVFIFPPSDEQLKSGTASVVCLLNNFYPREAKVQWKVDNALQSGNSQESVTEQDSKDSTYSLSSTLTLSKADYEKHKVYACEVTHQGLSSPVTKSFNRGEC

SEQ ID NO: 160 - protein, 223 aa, Artificial Sequence
  Synthetic Construct
EVQLVQSGAEVKKPGASVKVSCKASGYKFTDSEMHWVRQAPGQGLEWIGGVDPETEGAAYNQKFKGRATITRDTSTSTAYLELSSLRSEDTAVYYCTRGYDYDYALDYWGQGTLVTVSSASTKGPSVFPLAPSSKSTSGGTAALGCLVKDYFPEPVTVSWNSGALTSGVHTFPAVLQSSGLYSLSSVVTVPSSSLGTQTYICNVNHKPSNTKVDKKVEPKSCD